European Patent Application EP 4 379 727 A1, published June 5, 2024. Title: IMMUNE RECEPTOR-BARCODE ERROR CORRECTION. Applicant: Becton, Dickinson and Company. Application EP. The sequence listing filed with the application follows.

SEQUENCE LISTING (113 sequences)

SEQ ID NO: 1 - DNA, 20 bp, synthetic construct
  misc_feature 1..20: note = note="Description of Artificial Sequence: Synthetic Oligonucleotide or Polypeptide"
  source 1..20: mol_type = other DNA
aaaaaaaaaaaaaaaaaaaa

SEQ ID NO: 2 - DNA, 20 bp, synthetic construct
  misc_feature 1..20: note = note="Description of Artificial Sequence: Synthetic Oligonucleotide or Polypeptide"
  source 1..20: mol_type = other DNA
tttttttttttttttttttt

SEQ ID NO: 3-11 - skipped (9 entries)

SEQ ID NO: 12 - protein, 14 aa, synthetic construct
  REGION 1..14: note = note="Description of Artificial Sequence: Synthetic Oligonucleotide or Polypeptide"
CVVNGDGTASKLTF

SEQ ID NO: 13 - protein, 14 aa, synthetic construct
  REGION 1..14: note = note="Description of Artificial Sequence: Synthetic Oligonucleotide or Polypeptide"
CVVDGDGTASKLTF

SEQ ID NO: 14 - protein, 14 aa, synthetic construct
  REGION 1..14: note = note="Description of Artificial Sequence: Synthetic Oligonucleotide or Polypeptide"
CVVSGDGTASKLTF

SEQ ID NO: 15 - protein, 14 aa, synthetic construct
  REGION 1..14: note = note="Description of Artificial Sequence: Synthetic Oligonucleotide or Polypeptide"
CVVNGVGTASKLTF

SEQ ID NO: 16 - protein, 14 aa, synthetic construct
  REGION 1..14: note = note="Description of Artificial Sequence: Synthetic Oligonucleotide or Polypeptide"
CVVNGDGAASKLTF

SEQ ID NO: 17 - protein, 14 aa, synthetic construct
  REGION 1..14: note = note="Description of Artificial Sequence: Synthetic Oligonucleotide or Polypeptide"
CVVNGDGTAGKLTF

SEQ ID NO: 18 - protein, 14 aa, synthetic construct
  REGION 1..14: note = note="Description of Artificial Sequence: Synthetic Oligonucleotide or Polypeptide"
CVVNGDGTASRLTF

SEQ ID NO: 19 - protein, 14 aa, synthetic construct
  REGION 1..14: note = note="Description of Artificial Sequence: Synthetic Oligonucleotide or Polypeptide"
CVVNGDGTASKLAF

SEQ ID NO: 20 - protein, 14 aa, synthetic construct
  REGION 1..14: note = note="Description of Artificial Sequence: Synthetic Oligonucleotide or Polypeptide"
CVVNGDGTASKLTL

SEQ ID NO: 21 - protein, 14 aa, synthetic construct
  REGION 1..14: note = note="Description of Artificial Sequence: Synthetic Oligonucleotide or Polypeptide"
CVVNGDGTASKPTF

SEQ ID NO: 22 - protein, 14 aa, synthetic construct
  REGION 1..14: note = note="Description of Artificial Sequence: Synthetic Oligonucleotide or Polypeptide"
CVVNGDGTTSKLTF

SEQ ID NO: 23 - protein, 14 aa, synthetic construct
  REGION 1..14: note = note="Description of Artificial Sequence: Synthetic Oligonucleotide or Polypeptide"
CVVNEDGTASKLTF

SEQ ID NO: 24 - protein, 14 aa, synthetic construct
  REGION 1..14: note = note="Description of Artificial Sequence: Synthetic Oligonucleotide or Polypeptide"
CVANGDGTASKLTF

SEQ ID NO: 25 - protein, 14 aa, synthetic construct
  REGION 1..14: note = note="Description of Artificial Sequence: Synthetic Oligonucleotide or Polypeptide"
CVMNGDGTASKLTF

SEQ ID NO: 26 - protein, 14 aa, synthetic construct
  REGION 1..14: note = note="Description of Artificial Sequence: Synthetic Oligonucleotide or Polypeptide"
CAVNGDGTASKLTF

SEQ ID NO: 27 - protein, 14 aa, synthetic construct
  REGION 1..14: note = note="Description of Artificial Sequence: Synthetic Oligonucleotide or Polypeptide"
RVVNGDGTASKLTF

SEQ ID NO: 28 - protein, 13 aa, synthetic construct
  REGION 1..13: note = note="Description of Artificial Sequence: Synthetic Oligonucleotide or Polypeptide"
CAVHRGSQGNLIF

SEQ ID NO: 29 - protein, 13 aa, synthetic construct
  REGION 1..13: note = note="Description of Artificial Sequence: Synthetic Oligonucleotide or Polypeptide"
CAVHRGSQGNLIV

SEQ ID NO: 30 - protein, 13 aa, synthetic construct
  REGION 1..13: note = note="Description of Artificial Sequence: Synthetic Oligonucleotide or Polypeptide"
CAGESGDYQKVTF

SEQ ID NO: 31 - protein, 13 aa, synthetic construct
  REGION 1..13: note = note="Description of Artificial Sequence: Synthetic Oligonucleotide or Polypeptide"
CAGESGGYQKVTF

SEQ ID NO: 32 - protein, 13 aa, synthetic construct
  REGION 1..13: note = note="Description of Artificial Sequence: Synthetic Oligonucleotide or Polypeptide"
CAATESYGQNFVF

SEQ ID NO: 33 - protein, 15 aa, synthetic construct
  REGION 1..15: note = note="Description of Artificial Sequence: Synthetic Oligonucleotide or Polypeptide"
CLVGSLSGSARQLTF

SEQ ID NO: 34 - protein, 14 aa, synthetic construct
  REGION 1..14: note = note="Description of Artificial Sequence: Synthetic Oligonucleotide or Polypeptide"
CVVTASGGYQKVTF

SEQ ID NO: 35 - protein, 13 aa, synthetic construct
  REGION 1..13: note = note="Description of Artificial Sequence: Synthetic Oligonucleotide or Polypeptide"
CAVAPYGNNRLAF

SEQ ID NO: 36 - protein, 15 aa, synthetic construct
  REGION 1..15: note = note="Description of Artificial Sequence: Synthetic Oligonucleotide or Polypeptide"
CAVTRFSGGYNKLIF

SEQ ID NO: 37 - protein, 17 aa, synthetic construct
  REGION 1..17: note = note="Description of Artificial Sequence: Synthetic Oligonucleotide or Polypeptide"
CAVSKGARSGNTGKLIF

SEQ ID NO: 38 - protein, 10 aa, synthetic construct
  REGION 1..10: note = note="Description of Artificial Sequence: Synthetic Oligonucleotide or Polypeptide"
CALFNNDMRF

SEQ ID NO: 39 - protein, 13 aa, synthetic construct
  REGION 1..13: note = note="Description of Artificial Sequence: Synthetic Oligonucleotide or Polypeptide"
CALSPGGYQKVTF

SEQ ID NO: 40 - protein, 15 aa, synthetic construct
  REGION 1..15: note = note="Description of Artificial Sequence: Synthetic Oligonucleotide or Polypeptide"
CAGLKLETSGSRLTF

SEQ ID NO: 41 - protein, 11 aa, synthetic construct
  REGION 1..11: note = note="Description of Artificial Sequence: Synthetic Oligonucleotide or Polypeptide"
CAGGYGNKLVF

SEQ ID NO: 42 - protein, 16 aa, synthetic construct
  REGION 1..16: note = note="Description of Artificial Sequence: Synthetic Oligonucleotide or Polypeptide"
CAGARGSNFGNEKLTF

SEQ ID NO: 43 - protein, 12 aa, synthetic construct
  REGION 1..12: note = note="Description of Artificial Sequence: Synthetic Oligonucleotide or Polypeptide"
CAANNAGNVLTF

SEQ ID NO: 44 - protein, 15 aa, synthetic construct
  REGION 1..15: note = note="Description of Artificial Sequence: Synthetic Oligonucleotide or Polypeptide"
CAAPSLGGSARQLTF

SEQ ID NO: 45 - protein, 15 aa, synthetic construct
  REGION 1..15: note = "Description of Artificial Sequence: Synthetic Oligonucleotide or Polypeptide"
CAASIRGDSSYKLIF

SEQ ID NO: 46 - protein, 13 aa, synthetic construct
  REGION 1..13: note = "Description of Artificial Sequence: Synthetic Oligonucleotide or Polypeptide"
  REGION 7..8: note = Position that corresponds to a stop codon
CAASRADGNQFYF

SEQ ID NO: 47 - protein, 14 aa, synthetic construct
  REGION 1..14: note = note="Description of Artificial Sequence: Synthetic Oligonucleotide or Polypeptide"
CAASPMNRDDKIIF

SEQ ID NO: 48 - protein, 14 aa, synthetic construct
  REGION 1..14: note = note="Description of Artificial Sequence: Synthetic Oligonucleotide or Polypeptide"
CAASITDSWGKLQF

SEQ ID NO: 49 - protein, 13 aa, synthetic construct
  REGION 1..13: note = note="Description of Artificial Sequence: Synthetic Oligonucleotide or Polypeptide"
CVVSAKNTDKLIF

SEQ ID NO: 50 - protein, 12 aa, synthetic construct
  REGION 1..12: note = note="Description of Artificial Sequence: Synthetic Oligonucleotide or Polypeptide"
CAYRSSNYQLIW

SEQ ID NO: 51 - protein, 15 aa, synthetic construct
  REGION 1..15: note = note="Description of Artificial Sequence: Synthetic Oligonucleotide or Polypeptide"
CAVVPFGGGGNKLTF

SEQ ID NO: 52 - protein, 12 aa, synthetic construct
  REGION 1..12: note = note="Description of Artificial Sequence: Synthetic Oligonucleotide or Polypeptide"
CAGWSNDYKLSF

SEQ ID NO: 53 - protein, 13 aa, synthetic construct
  REGION 1..13: note = note="Description of Artificial Sequence: Synthetic Oligonucleotide or Polypeptide"
CAASGGSNYKLTF

SEQ ID NO: 54 - protein, 16 aa, synthetic construct
  REGION 1..16: note = note="Description of Artificial Sequence: Synthetic Oligonucleotide or Polypeptide"
CAMREGGGSNDYKLSF

SEQ ID NO: 55 - protein, 13 aa, synthetic construct
  REGION 1..13: note = note="Description of Artificial Sequence: Synthetic Oligonucleotide or Polypeptide"
CIRLPGNTGKLIF

SEQ ID NO: 56 - protein, 13 aa, synthetic construct
  REGION 1..13: note = note="Description of Artificial Sequence: Synthetic Oligonucleotide or Polypeptide"
CAYVAAAGNKLTF

SEQ ID NO: 57 - protein, 12 aa, synthetic construct
  REGION 1..12: note = note="Description of Artificial Sequence: Synthetic Oligonucleotide or Polypeptide"
CAGAPGSYIPTF

SEQ ID NO: 58 - DNA, 42 bp, synthetic construct
  misc_feature 1..42: note = note="Description of Artificial Sequence: Synthetic Oligonucleotide or Polypeptide"
  source 1..42: mol_type = other DNA
tgtgtggtgaacggagacggcactgccagtaaactcaccttt

SEQ ID NO: 59 - DNA, 42 bp, synthetic construct
  misc_feature 1..42: note = note="Description of Artificial Sequence: Synthetic Oligonucleotide or Polypeptide"
  source 1..42: mol_type = other DNA
tgtgtggtggacggagacggcactgctagtaaactcaccttt

SEQ ID NO: 60 - DNA, 42 bp, synthetic construct
  misc_feature 1..42: note = note="Description of Artificial Sequence: Synthetic Oligonucleotide or Polypeptide"
  source 1..42: mol_type = other DNA
tgtgtggtgagcggagacggcactgccagtaaactcaccttt

SEQ ID NO: 61 - DNA, 42 bp, synthetic construct
  misc_feature 1..42: note = note="Description of Artificial Sequence: Synthetic Oligonucleotide or Polypeptide"
  source 1..42: mol_type = other DNA
tgtgtggtgaacggagtcggcactgccagtaaactcaccttt

SEQ ID NO: 62 - DNA, 42 bp, synthetic construct
  misc_feature 1..42: note = note="Description of Artificial Sequence: Synthetic Oligonucleotide or Polypeptide"
  source 1..42: mol_type = other DNA
tgtgtggtgaacggagacggcgctgccagtaaactcaccttt

SEQ ID NO: 63 - DNA, 42 bp, synthetic construct
  misc_feature 1..42: note = note="Description of Artificial Sequence: Synthetic Oligonucleotide or Polypeptide"
  source 1..42: mol_type = other DNA
tgtgtggtgaacggagacggcactgccggtaaactcaccttt

SEQ ID NO: 64 - DNA, 42 bp, synthetic construct
  misc_feature 1..42: note = note="Description of Artificial Sequence: Synthetic Oligonucleotide or Polypeptide"
  source 1..42: mol_type = other DNA
tgtgtggtgaacggagacggcactgccagtagactcaccttt

SEQ ID NO: 65 - DNA, 42 bp, synthetic construct
  misc_feature 1..42: note = note="Description of Artificial Sequence: Synthetic Oligonucleotide or Polypeptide"
  source 1..42: mol_type = other DNA
tgtgtggtgaacggagacggcactgccagtaaactcgccttt

SEQ ID NO: 66 - DNA, 42 bp, synthetic construct
  misc_feature 1..42: note = note="Description of Artificial Sequence: Synthetic Oligonucleotide or Polypeptide"
  source 1..42: mol_type = other DNA
tgtgtggtgaacggagacggcactgccagtaaactcactttt

SEQ ID NO: 67 - DNA, 42 bp, synthetic construct
  misc_feature 1..42: note = note="Description of Artificial Sequence: Synthetic Oligonucleotide or Polypeptide"
  source 1..42: mol_type = other DNA
tgtgtggtgaacggagacggcactgccagtaaactcaccctt

SEQ ID NO: 68 - DNA, 42 bp, synthetic construct
  misc_feature 1..42: note = note="Description of Artificial Sequence: Synthetic Oligonucleotide or Polypeptide"
  source 1..42: mol_type = other DNA
tgtgtggtgaacggagacggcactgccagtaaacccaccttt

SEQ ID NO: 69 - DNA, 42 bp, synthetic construct
  misc_feature 1..42: note = note="Description of Artificial Sequence: Synthetic Oligonucleotide or Polypeptide"
  source 1..42: mol_type = other DNA
tgtgtggtgaacggagacggcactgccagcaaactcaccttt

SEQ ID NO: 70 - DNA, 42 bp, synthetic construct
  misc_feature 1..42: note = note="Description of Artificial Sequence: Synthetic Oligonucleotide or Polypeptide"
  source 1..42: mol_type = other DNA
tgtgtggtgaacggagacggcactaccagtaaactcaccttt

SEQ ID NO: 71 - DNA, 42 bp, synthetic construct
  misc_feature 1..42: note = note="Description of Artificial Sequence: Synthetic Oligonucleotide or Polypeptide"
  source 1..42: mol_type = other DNA
tgtgtggtgaacggagacggcacagccagtaaactcaccttt

SEQ ID NO: 72 - DNA, 42 bp, synthetic construct
  misc_feature 1..42: note = note="Description of Artificial Sequence: Synthetic Oligonucleotide or Polypeptide"
  source 1..42: mol_type = other DNA
tgtgtggtgaacgaagacggcactgccagtaaactcaccttt

SEQ ID NO: 73 - DNA, 42 bp, synthetic construct
  misc_feature 1..42: note = note="Description of Artificial Sequence: Synthetic Oligonucleotide or Polypeptide"
  source 1..42: mol_type = other DNA
tgtgtggcgaacggagacggcactgccagtaaactcaccttt

SEQ ID NO: 74 - DNA, 42 bp, synthetic construct
  misc_feature 1..42: note = note="Description of Artificial Sequence: Synthetic Oligonucleotide or Polypeptide"
  source 1..42: mol_type = other DNA
tgtgtgatgaacggagacggcactgccagtaaactcaccttt

SEQ ID NO: 75 - DNA, 42 bp, synthetic construct
  misc_feature 1..42: note = note="Description of Artificial Sequence: Synthetic Oligonucleotide or Polypeptide"
  source 1..42: mol_type = other DNA
tgtgcggtgaacggagacggcactgccagtaaactcaccttt

SEQ ID NO: 76 - DNA, 42 bp, synthetic construct
  misc_feature 1..42: note = note="Description of Artificial Sequence: Synthetic Oligonucleotide or Polypeptide"
  source 1..42: mol_type = other DNA
tgcgtggtgaacggagacggcactgccagtaaactcaccttt

SEQ ID NO: 77 - DNA, 42 bp, synthetic construct
  misc_feature 1..42: note = note="Description of Artificial Sequence: Synthetic Oligonucleotide or Polypeptide"
  source 1..42: mol_type = other DNA
cgtgtggtgaacggagacggcactgccagtaaactcaccttt

SEQ ID NO: 78 - DNA, 39 bp, synthetic construct
  misc_feature 1..39: note = note="Description of Artificial Sequence: Synthetic Oligonucleotide or Polypeptide"
  source 1..39: mol_type = other DNA
tgtgctgtccaccgaggaagccaaggaaatctcatcttt

SEQ ID NO: 79 - DNA, 39 bp, synthetic construct
  misc_feature 1..39: note = note="Description of Artificial Sequence: Synthetic Oligonucleotide or Polypeptide"
  source 1..39: mol_type = other DNA
tgtgctgtccaccgaggaagccaaggaaatctcatcgtt

SEQ ID NO: 80 - DNA, 39 bp, synthetic construct
  misc_feature 1..39: note = note="Description of Artificial Sequence: Synthetic Oligonucleotide or Polypeptide"
  source 1..39: mol_type = other DNA
tgtgcaggagaatctggggattaccagaaagttaccttt

SEQ ID NO: 81 - DNA, 39 bp, synthetic construct
  misc_feature 1..39: note = note="Description of Artificial Sequence: Synthetic Oligonucleotide or Polypeptide"
  source 1..39: mol_type = other DNA
tgtgcaggagaatctgggggttaccagaaagttaccttt

SEQ ID NO: 82 - DNA, 39 bp, synthetic construct
  misc_feature 1..39: note = note="Description of Artificial Sequence: Synthetic Oligonucleotide or Polypeptide"
  source 1..39: mol_type = other DNA
tgtgcagcaaccgagtcctatggtcagaattttgtcttt

SEQ ID NO: 83 - DNA, 39 bp, synthetic construct
  misc_feature 1..39: note = note="Description of Artificial Sequence: Synthetic Oligonucleotide or Polypeptide"
  source 1..39: mol_type = other DNA
tgtgcagcaacagagtcctatggtcagaattttgtcttt

SEQ ID NO: 84 - DNA, 45 bp, synthetic construct
  misc_feature 1..45: note = note="Description of Artificial Sequence: Synthetic Oligonucleotide or Polypeptide"
  source 1..45: mol_type = other DNA
tgcctcgtggggagcctttctggttctgcaaggcaactgaccttt

SEQ ID NO: 85 - DNA, 45 bp, synthetic construct
  misc_feature 1..45: note = note="Description of Artificial Sequence: Synthetic Oligonucleotide or Polypeptide"
  source 1..45: mol_type = other DNA
tgcctcgtggggagcctttccggttctgcaaggcaactgaccttt

SEQ ID NO: 86 - DNA, 42 bp, synthetic construct
  misc_feature 1..42: note = note="Description of Artificial Sequence: Synthetic Oligonucleotide or Polypeptide"
  source 1..42: mol_type = other DNA
tgtgtggtgaccgcttctgggggttaccagaaagttaccttt

SEQ ID NO: 87 - DNA, 39 bp, synthetic construct
  misc_feature 1..39: note = note="Description of Artificial Sequence: Synthetic Oligonucleotide or Polypeptide"
  source 1..39: mol_type = other DNA
tgtgctgtggccccctatgggaacaacagactcgctttt

SEQ ID NO: 88 - DNA, 45 bp, synthetic construct
  misc_feature 1..45: note = note="Description of Artificial Sequence: Synthetic Oligonucleotide or Polypeptide"
  source 1..45: mol_type = other DNA
tgtgctgtgactcggttttctggtggctacaataagctgattttt

SEQ ID NO: 89 - DNA, 51 bp, synthetic construct
  misc_feature 1..51: note = note="Description of Artificial Sequence: Synthetic Oligonucleotide or Polypeptide"
  source 1..51: mol_type = other DNA
tgtgctgtcagtaagggggctaggtctggcaacacaggcaaactaatcttt

SEQ ID NO: 90 - DNA, 30 bp, synthetic construct
  misc_feature 1..30: note = note="Description of Artificial Sequence: Synthetic Oligonucleotide or Polypeptide"
  source 1..30: mol_type = other DNA
tgtgctctgtttaacaatgacatgcgcttt

SEQ ID NO: 91 - DNA, 39 bp, synthetic construct
  misc_feature 1..39: note = note="Description of Artificial Sequence: Synthetic Oligonucleotide or Polypeptide"
  source 1..39: mol_type = other DNA
tgtgctctgtcccctgggggttaccagaaagttaccttt

SEQ ID NO: 92 - DNA, 45 bp, synthetic construct
  misc_feature 1..45: note = note="Description of Artificial Sequence: Synthetic Oligonucleotide or Polypeptide"
  source 1..45: mol_type = other DNA
tgtgcagggttaaaactagaaaccagtggctctaggttgaccttt

SEQ ID NO: 93 - DNA, 33 bp, synthetic construct
  misc_feature 1..33: note = note="Description of Artificial Sequence: Synthetic Oligonucleotide or Polypeptide"
  source 1..33: mol_type = other DNA
tgtgcaggggggtatggaaacaaactggtcttt

SEQ ID NO: 94 - DNA, 48 bp, synthetic construct
  misc_feature 1..48: note = note="Description of Artificial Sequence: Synthetic Oligonucleotide or Polypeptide"
  source 1..48: mol_type = other DNA
tgtgcaggagcgaggggatctaactttggaaatgagaaattaaccttt

SEQ ID NO: 95 - DNA, 36 bp, synthetic construct
  misc_feature 1..36: note = note="Description of Artificial Sequence: Synthetic Oligonucleotide or Polypeptide"
  source 1..36: mol_type = other DNA
tgtgcagctaataatgcaggcaacgtgctcaccttt

SEQ ID NO: 96 - DNA, 45 bp, synthetic construct
  misc_feature 1..45: note = note="Description of Artificial Sequence: Synthetic Oligonucleotide or Polypeptide"
  source 1..45: mol_type = other DNA
tgtgcagccccctccctggggggttctgcaaggcaactgaccttt

SEQ ID NO: 97 - DNA, 45 bp, synthetic construct
  misc_feature 1..45: note = note="Description of Artificial Sequence: Synthetic Oligonucleotide or Polypeptide"
  source 1..45: mol_type = other DNA
tgtgcagcaagtataaggggggatagcagctataaattgatcttc

SEQ ID NO: 98 - DNA, 40 bp, synthetic construct
  misc_feature 1..40: note = note="Description of Artificial Sequence: Synthetic Oligonucleotide or Polypeptide"
  source 1..40: mol_type = other DNA
tgtgcagcaagtagagccgaccggtaaccagttctatttt

SEQ ID NO: 99 - DNA, 42 bp, synthetic construct
  misc_feature 1..42: note = note="Description of Artificial Sequence: Synthetic Oligonucleotide or Polypeptide"
  source 1..42: mol_type = other DNA
tgtgcagcaagcccaatgaacagagatgacaagatcatcttt

SEQ ID NO: 100 - DNA, 42 bp, synthetic construct
  misc_feature 1..42: note = note="Description of Artificial Sequence: Synthetic Oligonucleotide or Polypeptide"
  source 1..42: mol_type = other DNA
tgtgcagcaagcataactgacagctgggggaaattgcagttt

SEQ ID NO: 101 - DNA, 39 bp, synthetic construct
  misc_feature 1..39: note = note="Description of Artificial Sequence: Synthetic Oligonucleotide or Polypeptide"
  source 1..39: mol_type = other DNA
tgtgtggtgagcgcgaaaaacaccgacaagctcatcttt

SEQ ID NO: 102 - DNA, 36 bp, synthetic construct
  misc_feature 1..36: note = note="Description of Artificial Sequence: Synthetic Oligonucleotide or Polypeptide"
  source 1..36: mol_type = other DNA
tgtgcttataggagtagcaactatcagttaatctgg

SEQ ID NO: 103 - DNA, 45 bp, synthetic construct
  misc_feature 1..45: note = note="Description of Artificial Sequence: Synthetic Oligonucleotide or Polypeptide"
  source 1..45: mol_type = other DNA
tgtgctgtggtccccttcgggggaggaggaaacaaactcaccttt

SEQ ID NO: 104 - DNA, 36 bp, synthetic construct
  misc_feature 1..36: note = note="Description of Artificial Sequence: Synthetic Oligonucleotide or Polypeptide"
  source 1..36: mol_type = other DNA
tgtgcaggatggtctaacgactacaagctcagcttt

SEQ ID NO: 105 - DNA, 39 bp, synthetic construct
  misc_feature 1..39: note = note="Description of Artificial Sequence: Synthetic Oligonucleotide or Polypeptide"
  source 1..39: mol_type = other DNA
tgtgcagcaagtggaggtagcaactataaactgacattt

SEQ ID NO: 106 - DNA, 48 bp, synthetic construct
  misc_feature 1..48: note = note="Description of Artificial Sequence: Synthetic Oligonucleotide or Polypeptide"
  source 1..48: mol_type = other DNA
tgtgcaatgagagagggcggtggttctaacgactacaagctcagcttt

SEQ ID NO: 107 - DNA, 39 bp, synthetic construct
  misc_feature 1..39: note = note="Description of Artificial Sequence: Synthetic Oligonucleotide or Polypeptide"
  source 1..39: mol_type = other DNA
tgcatccgcctgcctggcaacacaggcaaactaatcttt

SEQ ID NO: 108 - DNA, 39 bp, synthetic construct
  misc_feature 1..39: note = note="Description of Artificial Sequence: Synthetic Oligonucleotide or Polypeptide"
  source 1..39: mol_type = other DNA
tgtgcttatgtcgcagctgcaggcaacaagctaactttt

SEQ ID NO: 109 - DNA, 36 bp, synthetic construct
  misc_feature 1..36: note = note="Description of Artificial Sequence: Synthetic Oligonucleotide or Polypeptide"
  source 1..36: mol_type = other DNA
tgtgcaggagccccaggaagctacatacctacattt

SEQ ID NO: 110-113 - skipped (4 entries)